European Patent Application EP 4 253 959 A2, published October 4, 2023. Title: ANTI‐IDIOTYPIC ANTIBODIES DIRECTED TO THE ANTIGEN‐BINDING PORTION OF AN BCMA‐BINDING MOLECULE. Applicant: KITE PHARMA, INC. The sequence listing filed with the application follows.

SEQUENCE LISTING (129 sequences)

SEQ ID NO: 1-3 - skipped (3 entries)

SEQ ID NO: 4 - DNA, 426 bp, synthetic construct
  source 1..426: mol_type = other DNA
atggagactgggctgcgctggcttctcctggtcgctgtgctcaaaggtgtccagtgtcagcagcagctggaggagtccgggggaggcctggtcaagcctggaggaaccctgacactcacctgcacagcctctggattctccttcagtagcggccaatggatgtgttgggtccgccaggctccagggaaggggctggaattgatcgcatgcatttatactagtgctggtggtagcacacattacgcgagctgggcgacaggccgattcaccatctccaaaacctcgtcgaccacggtgactctgcaaatgaccagtctgacagccgcggacacggccacctatttctgtgcgagagatccctatcttcttagtgctggtcctgataataatttgtggggcccaggcaccctggtcgccgtctcctca

SEQ ID NO: 5 - DNA, 426 bp, synthetic construct
  misc_feature 1..426: note = source = /note="Description of Artificial Sequence: Synthetic polynucleotide"
  source 1..426: mol_type = other DNA
atggagactgggctgcgctggcttctcctggtcgctgtgctcaaaggtgtccagtgtcagcagcagctggaggagtccgggggaggcctggtcaagcctggaggaaccctgacactcacctgcacagcctctggattctccttcagtagcggccaaaggatgtgttgggtccgccaggctccagggaaggggctggaattgatcgcatgcatttatactagtgctggtggtagcacacattacgcgagctgggcgacaggccgattcaccatctccaaaacctcgtcgaccacggtgactctgcaaatgaccagtctgacagccgcggacacggccacctatttctgtgcgagagatccctatcttcttagtgctggtcctgataataatttgtggggcccaggcaccctggtcgccgtctcctca

SEQ ID NO: 6 - DNA, 417 bp, synthetic construct
  misc_feature 1..417: note = source = /note="Description of Artificial Sequence: Synthetic polynucleotide"
  source 1..417: mol_type = other DNA
atggagactgggctgcgctggcttctcctggtcgctgtgctcaaaggtgtccagtgtcaggagcgcctggtggagtccgggggaggcctggtccagcctgagggatccctgacactcacctgcacagcctctggactcaccctcagtaactactggctgtgctgggtccgccaggctccagggaaggggctggagtggatcgcatgcatttatactggtaattatggtagcgcttactacgcgaactgggtgaaaggccgattcaccatctccaaagcctcgtcgaccacggtgactctgcaaatgaccagtctgacagccgcggacacggccacctatttctgtgcgagagatccttatactctaaccaatgttgatgtcttatggggcccaggcaccctggtcaccgtctcctca

SEQ ID NO: 7 - DNA, 426 bp, synthetic construct
  misc_feature 1..426: note = source = /note="Description of Artificial Sequence: Synthetic polynucleotide"
  source 1..426: mol_type = other DNA
atggagactgggctgcgctggcttctcctggtcgctgtgctcaaaggtgtccagtgtcaggagcagttggaggagtccgggggagacctggtcaagcctggggcatccctgacactcacctgcacagcctctggattctccttcagtagcggctattggatatgttgggtccgccaggctccagggaaggggctggagtggatcgcatgcatttatactcgtagtggtggtagcactcactacgcgagctgggcgaaaggccgattcaccacctccaaaacctcgtcgaccacggtgactctgcaaatgaccagtctgacagccgcggacatggccacctatttctgtgcgagagatccctatgttcttagtgctggtcctgataatgttttgtggggcccaggcaccctggtcaccgtctcctca

SEQ ID NO: 8 - DNA, 426 bp, synthetic construct
  misc_feature 1..426: note = source = /note="Description of Artificial Sequence: Synthetic polynucleotide"
  source 1..426: mol_type = other DNA
atggagactgggctgcgctggcttctcctggtcgctgtgctcaaaggtgtccagtgtcaggagcagctggaggagtccgggggagacctggtcaagcctgagggatccctgacactcacctgcacagcctctggattctccttcagtagcgcctattggatatgttgggtccgccaggttccagggaaggggctggagtggatcgcatgcatttatactggtagtggtggtaggtctcactacgcgagctgggcgaaaggccgattcaccatctccaaaacctcgtcgaccacggtgactctgcaaatgaccagtctgacagccgcggacacggccacctatttctgtgcgagagatccctatattcttagtgctggtcctgataatgttttgtggggcccaggcaccctggtcaccgtctcctca

SEQ ID NO: 9 - DNA, 423 bp, synthetic construct
  misc_feature 1..423: note = source = /note="Description of Artificial Sequence: Synthetic polynucleotide"
  source 1..423: mol_type = other DNA
atggagactgggctgcgctggcttctcctggtcgctgtgctcaaaggtgtccagtgtcaggagcagctggtggagtccgggggaggcctggtccagcctgagggatccctgacactcacctgcacagcctctggattctccttcagtctcagcaattggatatgctgggtccgccaggctccagggaaggggctggagtgggtcgcatgcatttatgttagtgtgagcggtaacactcgctacgcgagctgggcgaaaggccgattcaccatctccgaaacctcgtcgaccacggtgactctgcaaatgaccggtctgacagccgcggacacggccacctatttctgtgcgcgagatccatttagccttgtgagtgttgatcgttccttatggggcccaggcaccctggtcaccgtctcctca

SEQ ID NO: 10 - DNA, 417 bp, synthetic construct
  misc_feature 1..417: note = source = /note="Description of Artificial Sequence: Synthetic polynucleotide"
  source 1..417: mol_type = other DNA
atggagactgggctgcgctggcttctcctggtcgctgtgctcaaaggtgtccagtgtcagtcgttggaggagtccgggggagacctggtcaagcctgagggatccctgacactcacctgcacagcctctggattctccttcagtagcagctactggatatgctgggtccgccaggctccagggaaggggctggagtggatcgcatgcatttataccgctaacagtggtcgcactgtctacgcgagctgggcgaagggccgattcaccatctccaaaacctcgtcgaccacggtgactctgcagctgcccagtctgacagccgcggacacggccacctatttctgtgcgagagatatttatgtgcttactactactgataacttgtggggcccaggcaccctggtcaccgtctcctca

SEQ ID NO: 11 - protein, 142 aa, synthetic construct
  REGION 1..142: note = source = /note="Description of Artificial Sequence: Synthetic polypeptide"
METGLRWLLLVAVLKGVQCQQQLEESGGGLVKPGGTLTLTCTASGFSFSSGQWMCWVRQAPGKGLELIACIYTSAGGSTHYASWATGRFTISKTSSTTVTLQMTSLTAADTATYFCARDPYLLSAGPDNNLWGPGTLVAVSS

SEQ ID NO: 12 - protein, 142 aa, synthetic construct
  REGION 1..142: note = source = /note="Description of Artificial Sequence: Synthetic polypeptide"
METGLRWLLLVAVLKGVQCQQQLEESGGGLVKPGGTLTLTCTASGFSFSSGQRMCWVRQAPGKGLELIACIYTSAGGSTHYASWATGRFTISKTSSTTVTLQMTSLTAADTATYFCARDPYLLSAGPDNNLWGPGTLVAVSS

SEQ ID NO: 13 - protein, 139 aa, synthetic construct
  REGION 1..139: note = source = /note="Description of Artificial Sequence: Synthetic polypeptide"
METGLRWLLLVAVLKGVQCQERLVESGGGLVQPEGSLTLTCTASGLTLSNYWLCWVRQAPGKGLEWIACIYTGNYGSAYYANWVKGRFTISKASSTTVTLQMTSLTAADTATYFCARDPYTLTNVDVLWGPGTLVTVSS

SEQ ID NO: 14 - protein, 142 aa, synthetic construct
  REGION 1..142: note = source = /note="Description of Artificial Sequence: Synthetic polypeptide"
METGLRWLLLVAVLKGVQCQEQLEESGGDLVKPGASLTLTCTASGFSFSSGYWICWVRQAPGKGLEWIACIYTRSGGSTHYASWAKGRFTTSKTSSTTVTLQMTSLTAADMATYFCARDPYVLSAGPDNVLWGPGTLVTVSS

SEQ ID NO: 15 - protein, 142 aa, synthetic construct
  REGION 1..142: note = source = /note="Description of Artificial Sequence: Synthetic polypeptide"
METGLRWLLLVAVLKGVQCQEQLEESGGDLVKPEGSLTLTCTASGFSFSSAYWICWVRQVPGKGLEWIACIYTGSGGRSHYASWAKGRFTISKTSSTTVTLQMTSLTAADTATYFCARDPYILSAGPDNVLWGPGTLVTVSS

SEQ ID NO: 16 - protein, 141 aa, synthetic construct
  REGION 1..141: note = source = /note="Description of Artificial Sequence: Synthetic polypeptide"
METGLRWLLLVAVLKGVQCQEQLVESGGGLVQPEGSLTLTCTASGFSFSLSNWICWVRQAPGKGLEWVACIYVSVSGNTRYASWAKGRFTISETSSTTVTLQMTGLTAADTATYFCARDPFSLVSVDRSLWGPGTLVTVSS

SEQ ID NO: 17 - protein, 139 aa, synthetic construct
  REGION 1..139: note = source = /note="Description of Artificial Sequence: Synthetic polypeptide"
METGLRWLLLVAVLKGVQCQSLEESGGDLVKPEGSLTLTCTASGFSFSSSYWICWVRQAPGKGLEWIACIYTANSGRTVYASWAKGRFTISKTSSTTVTLQLPSLTAADTATYFCARDIYVLTTTDNLWGPGTLVTVSS

SEQ ID NO: 18 - DNA, 396 bp, synthetic construct
  misc_feature 1..396: note = source = /note="Description of Artificial Sequence: Synthetic polynucleotide"
  source 1..396: mol_type = other DNA
atggacacgagggcccccactcagctgctggggctcctgctgctctggctcccagatgccagatgtgcgcttgtgatgacccagactccatcccctgtgtctgcagctgtgggaggcacagtcaccatcaattgccaggccagtcagagcattggtagcgactttacctggtggcagcagaaaccagggcagcctcccaaactcctgatctactgggcatccactctggcatctggggtctcatcgcggttcaaaggcagtggatctgggacacagttcactctcaccatcagcgacctggagtgtgacgatgctgccacttactactgtgcaggctatgtaagttatagtgatgatggtaatgctttcggcggagggaccgaggtggtggtcaaa

SEQ ID NO: 19 - DNA, 396 bp, synthetic construct; identical to SEQ ID NO: 18
  misc_feature 1..396: note = source = /note="Description of Artificial Sequence: Synthetic polynucleotide"
  source 1..396: mol_type = other DNA

SEQ ID NO: 20 - DNA, 396 bp, synthetic construct
  misc_feature 1..396: note = source = /note="Description of Artificial Sequence: Synthetic polynucleotide"
  source 1..396: mol_type = other DNA
atggacacgagggcccccactcagctgctggggctcctgctgctctggctcccaggtgccagatgtgcccttgtgatgacccagactccatcccccgtgtctgcagctgtgggaggcacagtcaccatcaattgccaggccagtcagagcattggtagcgacttagcctggtatcagcagagaccagggcagcctcccaagctcctgatctactgggcatccactctggcatctggggtcccatcgcggttcagcggcagtggatctgggacacagttcactctcaccatcagcgacctggagtgtgacgatgccgccacttactactgtacaggctatataagttataatgatgataatgccgcgttcggcggagggaccgaggtggtggtcaaa

SEQ ID NO: 21 - DNA, 396 bp, synthetic construct
  misc_feature 1..396: note = source = /note="Description of Artificial Sequence: Synthetic polynucleotide"
  source 1..396: mol_type = other DNA
atggacacgagggcccccactcagctgctggggctcctgctgctctggctcccagatgccagatgtgcgcttgtgatgacccagactccatcccctgtgtctgcagctgtgggaggcacggtcaccatcaattgccaggccagtgagagcattggtagcgacttgggctggtatcagcagaaaccagggcagcctcccaaattcctgatctactgggcatccactttggtatctggggtcccatcgcggttcgaaggcagtggatctgggacacagttcactctcaccatcagcgacctggagtgtgacgatgctgccacttactactgtgcaggctatgaaagtttgagtaatgatggtaatgctttcggcggagggaccgaggtggtggtcaaa

SEQ ID NO: 22 - DNA, 396 bp, synthetic construct
  misc_feature 1..396: note = source = /note="Description of Artificial Sequence: Synthetic polynucleotide"
  source 1..396: mol_type = other DNA
atggacacgagggcccccactcagctgctggggctcctgctgctctggctcccagatgccagatgtgcgcttgtgatgacccagactccatcccctgtgtctgcagctgtgggaggcacagtcaccatcaattgccaggccagtcagagcattggtagcgacttaggctggtttcagcagaaaccagggcagcctcccaaactcctgatctactgggcatccactctggcatctggggtcccatcgcggttcgaaggcagtggatctgggacacagttcactctcaccatcagcgacctggagtgtgacgatgctgccacttactactgtgcaggctatgaaagtttgagtaatgatggtaatgctttcggcggagggaccgaggtggtggtcaaa

SEQ ID NO: 23 - DNA, 396 bp, synthetic construct
  misc_feature 1..396: note = source = /note="Description of Artificial Sequence: Synthetic polynucleotide"
  source 1..396: mol_type = other DNA
atggacacgagggcccccactcagctgctggggctcctgctgctctggctcccagatgccagatgtgcgcttgtgatgacccagactccatcccccgtgtctgcagctgtgggaggcacagtcaccatcaattgccaggccagtcagagcattggtagcgacttatcctggtttcagcagaaaccagggcagcctcccaagctcctgatgtactgggcatccagtctggcatctggggtcccatcgcggttcaaaggcagcggatctgggacacagttcactctcaccatcagcgacctggagtgtgacgatgctgccacttactactgtgcaggctatgtaaattataataatgatgatgctgctttcggcggagggaccgaggtggtggtcaaa

SEQ ID NO: 24 - DNA, 396 bp, synthetic construct
  misc_feature 1..396: note = source = /note="Description of Artificial Sequence: Synthetic polynucleotide"
  source 1..396: mol_type = other DNA
atggacacgagggcccccactcagctgctggggctcctgctgctctggctcccagatgccagatgtgcgcttgtgatgacccaggctccatcccctgtgtctgcagctgtgggaggcacagtcaccatcagttgccaggccagtcagcccattggtagcgacttagtttggtatcagcagaaaccagggcagcctcccaagctcctgatctattatgcatccgatctggcatctggggtcccatcgcggttcaaaggcagtggatctgggacacgattcactctcaccattagtggcgtggagtgtgacgatgctgccacttactactgtgcaggctataaaaattatgatcatgatgattgtggtttcggcggagggaccgaggtggtggtcaaa

SEQ ID NO: 25 - protein, 132 aa, synthetic construct
  REGION 1..132: note = source = /note="Description of Artificial Sequence: Synthetic polypeptide"
MDTRAPTQLLGLLLLWLPDARCALVMTQTPSPVSAAVGGTVTINCQASQSIGSDFTWWQQKPGQPPKLLIYWASTLASGVSSRFKGSGSGTQFTLTISDLECDDAATYYCAGYVSYSDDGNAFGGGTEVVVK

SEQ ID NO: 26 - protein, 132 aa, synthetic construct; identical to SEQ ID NO: 25
  REGION 1..132: note = source = /note="Description of Artificial Sequence: Synthetic polypeptide"

SEQ ID NO: 27 - protein, 132 aa, synthetic construct
  REGION 1..132: note = source = /note="Description of Artificial Sequence: Synthetic polypeptide"
MDTRAPTQLLGLLLLWLPGARCALVMTQTPSPVSAAVGGTVTINCQASQSIGSDLAWYQQRPGQPPKLLIYWASTLASGVPSRFSGSGSGTQFTLTISDLECDDAATYYCTGYISYNDDNAAFGGGTEVVVK

SEQ ID NO: 28 - protein, 132 aa, synthetic construct
  REGION 1..132: note = source = /note="Description of Artificial Sequence: Synthetic polypeptide"
MDTRAPTQLLGLLLLWLPDARCALVMTQTPSPVSAAVGGTVTINCQASESIGSDLGWYQQKPGQPPKFLIYWASTLVSGVPSRFEGSGSGTQFTLTISDLECDDAATYYCAGYESLSNDGNAFGGGTEVVVK

SEQ ID NO: 29 - protein, 132 aa, synthetic construct
  REGION 1..132: note = source = /note="Description of Artificial Sequence: Synthetic polypeptide"
MDTRAPTQLLGLLLLWLPDARCALVMTQTPSPVSAAVGGTVTINCQASQSIGSDLGWFQQKPGQPPKLLIYWASTLASGVPSRFEGSGSGTQFTLTISDLECDDAATYYCAGYESLSNDGNAFGGGTEVVVK

SEQ ID NO: 30 - protein, 132 aa, synthetic construct
  REGION 1..132: note = source = /note="Description of Artificial Sequence: Synthetic polypeptide"
MDTRAPTQLLGLLLLWLPDARCALVMTQTPSPVSAAVGGTVTINCQASQSIGSDLSWFQQKPGQPPKLLMYWASSLASGVPSRFKGSGSGTQFTLTISDLECDDAATYYCAGYVNYNNDDAAFGGGTEVVVK

SEQ ID NO: 31 - protein, 132 aa, synthetic construct
  REGION 1..132: note = source = /note="Description of Artificial Sequence: Synthetic polypeptide"
MDTRAPTQLLGLLLLWLPDARCALVMTQAPSPVSAAVGGTVTISCQASQPIGSDLVWYQQKPGQPPKLLIYYASDLASGVPSRFKGSGSGTRFTLTISGVECDDAATYYCAGYKNYDHDDCGFGGGTEVVVK

SEQ ID NO: 32 - protein, 11 aa, synthetic construct
  REGION 1..11: note = source = /note="Description of Artificial Sequence: Synthetic peptide"
QASQSIGSDFT

SEQ ID NO: 33 - protein, 11 aa, synthetic construct
  REGION 1..11: note = source = /note="Description of Artificial Sequence: Synthetic peptide"
QASQSIGSDLA

SEQ ID NO: 34 - protein, 11 aa, synthetic construct
  REGION 1..11: note = source = /note="Description of Artificial Sequence: Synthetic peptide"
QASESIGSDLG

SEQ ID NO: 35 - protein, 11 aa, synthetic construct
  REGION 1..11: note = source = /note="Description of Artificial Sequence: Synthetic peptide"
QASQSIGSDLG

SEQ ID NO: 36 - protein, 11 aa, synthetic construct
  REGION 1..11: note = source = /note="Description of Artificial Sequence: Synthetic peptide"
QASQSIGSDLS

SEQ ID NO: 37 - protein, 11 aa, synthetic construct
  REGION 1..11: note = source = /note="Description of Artificial Sequence: Synthetic peptide"
QASQPIGSDLV

SEQ ID NO: 38 - protein, 8 aa, synthetic construct
  REGION 1..8: note = source = /note="Description of Artificial Sequence: Synthetic peptide"
GFSFSSGQ

SEQ ID NO: 39 - protein, 6 aa, synthetic construct
  REGION 1..6: note = source = /note="Description of Artificial Sequence: Synthetic peptide"
SGQRMC

SEQ ID NO: 40 - protein, 5 aa, synthetic construct
  REGION 1..5: note = source = /note="Description of Artificial Sequence: Synthetic peptide"
NYWLC

SEQ ID NO: 41 - protein, 6 aa, synthetic construct
  REGION 1..6: note = source = /note="Description of Artificial Sequence: Synthetic peptide"
SGYWIC

SEQ ID NO: 42 - protein, 6 aa, synthetic construct
  REGION 1..6: note = source = /note="Description of Artificial Sequence: Synthetic peptide"
SAYWIC

SEQ ID NO: 43 - protein, 6 aa, synthetic construct
  REGION 1..6: note = source = /note="Description of Artificial Sequence: Synthetic peptide"
LSNWIC

SEQ ID NO: 44 - protein, 7 aa, synthetic construct
  REGION 1..7: note = source = /note="Description of Artificial Sequence: Synthetic peptide"
WASTLAS

SEQ ID NO: 45 - protein, 7 aa, synthetic construct
  REGION 1..7: note = source = /note="Description of Artificial Sequence: Synthetic peptide"
WASTLVS

SEQ ID NO: 46 - protein, 7 aa, synthetic construct
  REGION 1..7: note = source = /note="Description of Artificial Sequence: Synthetic peptide"
WASSLAS

SEQ ID NO: 47 - protein, 7 aa, synthetic construct
  REGION 1..7: note = source = /note="Description of Artificial Sequence: Synthetic peptide"
YASDLAS

SEQ ID NO: 48 - protein, 17 aa, synthetic construct
  REGION 1..17: note = source = /note="Description of Artificial Sequence: Synthetic peptide"
CIYTSAGGSTHYASWAT

SEQ ID NO: 49 - protein, 17 aa, synthetic construct
  REGION 1..17: note = source = /note="Description of Artificial Sequence: Synthetic peptide"
CIYTGNYGSAYYANWVK

SEQ ID NO: 50 - protein, 17 aa, synthetic construct
  REGION 1..17: note = source = /note="Description of Artificial Sequence: Synthetic peptide"
CIYTRSGGSTHYASWAK

SEQ ID NO: 51 - protein, 17 aa, synthetic construct
  REGION 1..17: note = source = /note="Description of Artificial Sequence: Synthetic peptide"
CIYTGSGGRSHYASWAK

SEQ ID NO: 52 - protein, 17 aa, synthetic construct
  REGION 1..17: note = source = /note="Description of Artificial Sequence: Synthetic peptide"
CIYVSVSGNTRYASWAK

SEQ ID NO: 53 - protein, 17 aa, synthetic construct
  REGION 1..17: note = source = /note="Description of Artificial Sequence: Synthetic peptide"
CIYTANSGRTVYASWAK

SEQ ID NO: 54 - protein, 12 aa, synthetic construct
  REGION 1..12: note = source = /note="Description of Artificial Sequence: Synthetic peptide"
AGYVSYSDDGNA

SEQ ID NO: 55 - protein, 12 aa, synthetic construct
  REGION 1..12: note = source = /note="Description of Artificial Sequence: Synthetic peptide"
TGYISYNDDNAA

SEQ ID NO: 56 - protein, 12 aa, synthetic construct
  REGION 1..12: note = source = /note="Description of Artificial Sequence: Synthetic peptide"
AGYESLSNDGNA

SEQ ID NO: 57 - protein, 12 aa, synthetic construct
  REGION 1..12: note = source = /note="Description of Artificial Sequence: Synthetic peptide"
AGYVNYNNDDAA

SEQ ID NO: 58 - protein, 12 aa, synthetic construct
  REGION 1..12: note = source = /note="Description of Artificial Sequence: Synthetic peptide"
AGYKNYDHDDCG

SEQ ID NO: 59 - protein, 13 aa, synthetic construct
  REGION 1..13: note = source = /note="Description of Artificial Sequence: Synthetic peptide"
DPYLLSAGPDNNL

SEQ ID NO: 60 - protein, 11 aa, synthetic construct
  REGION 1..11: note = source = /note="Description of Artificial Sequence: Synthetic peptide"
DPYTLTNVDVL

SEQ ID NO: 61 - protein, 13 aa, synthetic construct
  REGION 1..13: note = source = /note="Description of Artificial Sequence: Synthetic peptide"
DPYVLSAGPDNVL

SEQ ID NO: 62 - protein, 13 aa, synthetic construct
  REGION 1..13: note = source = /note="Description of Artificial Sequence: Synthetic peptide"
DPYILSAGPDNVL

SEQ ID NO: 63 - protein, 12 aa, synthetic construct
  REGION 1..12: note = source = /note="Description of Artificial Sequence: Synthetic peptide"
DPFSLVSVDRSL

SEQ ID NO: 64 - protein, 11 aa, synthetic construct
  REGION 1..11: note = source = /note="Description of Artificial Sequence: Synthetic peptide"
DIYVLTTTDNL

SEQ ID NO: 65 - protein, 8 aa, synthetic construct
  REGION 1..8: note = source = /note="Description of Artificial Sequence: Synthetic peptide"
GFSFSSGY

SEQ ID NO: 66 - protein, 8 aa, synthetic construct
  REGION 1..8: note = source = /note="Description of Artificial Sequence: Synthetic peptide"
GFSFSSAY

SEQ ID NO: 67 - protein, 8 aa, synthetic construct
  REGION 1..8: note = source = /note="Description of Artificial Sequence: Synthetic peptide"
GFSFSLSN

SEQ ID NO: 68 - protein, 6 aa, synthetic construct
  REGION 1..6: note = source = /note="Description of Artificial Sequence: Synthetic peptide"
YTSAGG

SEQ ID NO: 69 - protein, 6 aa, synthetic construct
  REGION 1..6: note = source = /note="Description of Artificial Sequence: Synthetic peptide"
YTGNYG

SEQ ID NO: 70 - protein, 6 aa, synthetic construct
  REGION 1..6: note = source = /note="Description of Artificial Sequence: Synthetic peptide"
YTRSGG

SEQ ID NO: 71 - protein, 6 aa, synthetic construct
  REGION 1..6: note = source = /note="Description of Artificial Sequence: Synthetic peptide"
YTGSGG

SEQ ID NO: 72 - protein, 6 aa, synthetic construct
  REGION 1..6: note = source = /note="Description of Artificial Sequence: Synthetic peptide"
YVSVSG

SEQ ID NO: 73 - protein, 6 aa, synthetic construct
  REGION 1..6: note = source = /note="Description of Artificial Sequence: Synthetic peptide"
YTANSG

SEQ ID NO: 74-83 - skipped (10 entries)

SEQ ID NO: 84 - protein, 6 aa, synthetic construct
  REGION 1..6: note = source = /note="Description of Artificial Sequence: Synthetic peptide"
SSYWIC

SEQ ID NO: 85 - protein, 8 aa, synthetic construct
  REGION 1..8: note = source = /note="Description of Artificial Sequence: Synthetic peptide"
GFSFSSSY

SEQ ID NO: 86 - DNA, 420 bp, synthetic construct
  misc_feature 1..420: note = source = /note="Description of Artificial Sequence: Synthetic polynucleotide"
  source 1..420: mol_type = other DNA
atggagactgggctgcgctggcttctcctggtcgctgtgctcaaaggtgtccagtgtcagtcgttggaggagtccgggggagccctggtcaagcctggggcatccctggcactcacctgcacagcctctggattctccttcaatctcaggcactacatgtgctgggtccgccaggctccggggaaggggctggagtggatcggatgcgttcatggtggtagtagtggtggcacttactacgcgagctggacgaaaggccgattcaccatatccaaaacctcgtcgaccacggtgactctgcaaatgaccagtctgacagccgcggacacggccacttatttctgtgcgagagaggatgatattatgatggccggagaatttagcttgtggggcccaggcaccctggtcaccgtctcctca

SEQ ID NO: 87 - DNA, 420 bp, synthetic construct
  misc_feature 1..420: note = source = /note="Description of Artificial Sequence: Synthetic polynucleotide"
  source 1..420: mol_type = other DNA
atggagactgggctgcgctggcttctcctggtcgctgtgctcaaaggtgtccagtgtcagtcgttggaggagtccgggggagacctggtcaagcctggggcatccctgacactcacctgcacagcctctggattctccttcaatctcaggcactacatgtgctgggtccgccaggctccggggaaggggctggagtggatcggatgcgttcatggtggtagtagtagtggcacttactacgcgagctgggcgaaaggccgattcaccatatccaaaacctcgtcgaccacggtgactctgcaaatgaccagtctgacagccgcggacacggccacttacttctgtacgagagaggatgatattatgatggccggagagtttggcttgtggggcccaggcaccctggtcaccgtctcctca

SEQ ID NO: 88 - DNA, 420 bp, synthetic construct
  misc_feature 1..420: note = source = /note="Description of Artificial Sequence: Synthetic polynucleotide"
  source 1..420: mol_type = other DNA
atggagactgggctgcgctggcttctcctggtcgctgtgctcaaaggtgtccagtgtcaggagcagctggtggagtccaggggaggcctggtcaagcctgggggatccctgacactcacctgcaaagcctctggattctccttcagtaccggctactacgcgtgctgggtccgccaggctccagggaaggggctggaattgagcgcatgcgttgatactggtagtggtgacactttctacgcgagctgggcgagaggccgattcaccatctccaaaacctcgtcatccacggtgactctgcaaatgaccagtctgacagttgcggacacggccacctatttctgtgcgaggacggcgctagtgatgactgatttctactttaacttgtggggcccaggcaccctgaccaccgtctcctca

SEQ ID NO: 89 - protein, 140 aa, synthetic construct
  REGION 1..140: note = source = /note="Description of Artificial Sequence: Synthetic polypeptide"
METGLRWLLLVAVLKGVQCQSLEESGGALVKPGASLALTCTASGFSFNLRHYMCWVRQAPGKGLEWIGCVHGGSSGGTYYASWTKGRFTISKTSSTTVTLQMTSLTAADTATYFCAREDDIMMAGEFSLWGPGTLVTVSS

SEQ ID NO: 90 - protein, 140 aa, synthetic construct
  REGION 1..140: note = source = /note="Description of Artificial Sequence: Synthetic polypeptide"
METGLRWLLLVAVLKGVQCQSLEESGGDLVKPGASLTLTCTASGFSFNLRHYMCWVRQAPGKGLEWIGCVHGGSSSGTYYASWAKGRFTISKTSSTTVTLQMTSLTAADTATYFCTREDDIMMAGEFGLWGPGTLVTVSS

SEQ ID NO: 91 - protein, 140 aa, synthetic construct
  REGION 1..140: note = source = /note="Description of Artificial Sequence: Synthetic polypeptide"
METGLRWLLLVAVLKGVQCQEQLVESRGGLVKPGGSLTLTCKASGFSFSTGYYACWVRQAPGKGLELSACVDTGSGDTFYASWARGRFTISKTSSSTVTLQMTSLTVADTATYFCARTALVMTDFYFNLWGPGTLTTVSS

SEQ ID NO: 92 - DNA, 396 bp, synthetic construct
  misc_feature 1..396: note = source = /note="Description of Artificial Sequence: Synthetic polynucleotide"
  source 1..396: mol_type = other DNA
atggacacgagggcccccactcagctgctggggctcctactgctctggctcccaggtgccagatgtgctgacattgtgatgacccagactccatcctccgtggaggcatctgtgggaggcacagtcaccatcaagtgccaggccagtgaggacattgaaagctacttagtctggtatcagcagaaaccagggcaacctcccaagctcctgatctaccaggcatccaatctggcctctggggtcccatcgcggttctacggcagtggatctgggacacagttcactctcaccatcagcgacctggagtgtgccgatgcttccacttactactgtcaaagttatgttgaaggtggtgttgatgttgttttcggcggagggaccgaggtggtggtcaaa

SEQ ID NO: 93 - DNA, 396 bp, synthetic construct
  misc_feature 1..396: note = source = /note="Description of Artificial Sequence: Synthetic polynucleotide"
  source 1..396: mol_type = other DNA
atggacacgagggcccccactcagctgctggggctcctactgctctggctcccaggtgccagatgtggtgacattgtgatgacccagactccatcctccgtgtctgaacctgtgggaggcacagtcaccatcaagtgccaggccagtgaggacattgaaagctatttagtctggtatcagcagaaaccagggcagcctcccaaactcctgatctaccaggcatccaatctggcctctggggtcccatcgcggttcagcggcagtggatctgggacagagtacactctcaccatcagcgacctggagtgtgccgatgctgccacttactactgtcaaagttatattgaaggtggtgttgatgttgttttcggcggagggaccgaggtggtggtcaaa

SEQ ID NO: 94 - DNA, 396 bp, synthetic construct
  misc_feature 1..396: note = source = /note="Description of Artificial Sequence: Synthetic polynucleotide"
  source 1..396: mol_type = other DNA
atggacacgagggcccccactcagctgctggggctcctgctgctctggctcccaggtgccagatgtgcccttgtgatgacccagactccagcctccgtggaggcagctgtgggaggcacagtcaccatcaattgccaggccagtcagtggattagcaatgaattatcctggtatcagcagaaaccagggcagcctcccaagctcctgatctatctggcatctactctggcatctggggtcccatcgcggttcaaaggcagtggatctgggacagagttcactctcaccatcagcgacctggagtgtgccgatgctgccacttactactgtcaacagggttataatataggccatcttgataatgctttcggcggagggaccgaggtggtggtcaaa

SEQ ID NO: 95 - protein, 132 aa, synthetic construct
  REGION 1..132: note = source = /note="Description of Artificial Sequence: Synthetic polypeptide"
MDTRAPTQLLGLLLLWLPGARCADIVMTQTPSSVEASVGGTVTIKCQASEDIESYLVWYQQKPGQPPKLLIYQASNLASGVPSRFYGSGSGTQFTLTISDLECADASTYYCQSYVEGGVDVVFGGGTEVVVK

SEQ ID NO: 96 - protein, 132 aa, synthetic construct
  REGION 1..132: note = source = /note="Description of Artificial Sequence: Synthetic polypeptide"
MDTRAPTQLLGLLLLWLPGARCGDIVMTQTPSSVSEPVGGTVTIKCQASEDIESYLVWYQQKPGQPPKLLIYQASNLASGVPSRFSGSGSGTEYTLTISDLECADAATYYCQSYIEGGVDVVFGGGTEVVVK

SEQ ID NO: 97 - protein, 132 aa, synthetic construct
  REGION 1..132: note = source = /note="Description of Artificial Sequence: Synthetic polypeptide"
MDTRAPTQLLGLLLLWLPGARCALVMTQTPASVEAAVGGTVTINCQASQWISNELSWYQQKPGQPPKLLIYLASTLASGVPSRFKGSGSGTEFTLTISDLECADAATYYCQQGYNIGHLDNAFGGGTEVVVK

SEQ ID NO: 98 - protein, 11 aa, synthetic construct
  REGION 1..11: note = source = /note="Description of Artificial Sequence: Synthetic peptide"
QASEDIESYLV

SEQ ID NO: 99 - protein, 11 aa, synthetic construct
  REGION 1..11: note = source = /note="Description of Artificial Sequence: Synthetic peptide"
QASQWISNELS

SEQ ID NO: 100 - protein, 7 aa, synthetic construct
  REGION 1..7: note = source = /note="Description of Artificial Sequence: Synthetic peptide"
QASNLAS

SEQ ID NO: 101 - protein, 7 aa, synthetic construct
  REGION 1..7: note = source = /note="Description of Artificial Sequence: Synthetic peptide"
LASTLAS

SEQ ID NO: 102 - protein, 11 aa, synthetic construct
  REGION 1..11: note = source = /note="Description of Artificial Sequence: Synthetic peptide"
QSYVEGGVDVV

SEQ ID NO: 103 - protein, 11 aa, synthetic construct
  REGION 1..11: note = source = /note="Description of Artificial Sequence: Synthetic peptide"
QSYIEGGVDVV

SEQ ID NO: 104 - protein, 12 aa, synthetic construct
  REGION 1..12: note = source = /note="Description of Artificial Sequence: Synthetic peptide"
QQGYNIGHLDNA

SEQ ID NO: 105 - protein, 6 aa, synthetic construct
  REGION 1..6: note = source = /note="Description of Artificial Sequence: Synthetic peptide"
LRHYMC

SEQ ID NO: 106 - protein, 6 aa, synthetic construct
  REGION 1..6: note = source = /note="Description of Artificial Sequence: Synthetic peptide"
TGYYAC

SEQ ID NO: 107 - protein, 17 aa, synthetic construct
  REGION 1..17: note = source = /note="Description of Artificial Sequence: Synthetic peptide"
CVHGGSSGGTYYASWTK

SEQ ID NO: 108 - protein, 17 aa, synthetic construct
  REGION 1..17: note = source = /note="Description of Artificial Sequence: Synthetic peptide"
CVHGGSSSGTYYASWAK

SEQ ID NO: 109 - protein, 16 aa, synthetic construct
  REGION 1..16: note = source = /note="Description of Artificial Sequence: Synthetic peptide"
CVDTGSGDTFYASWAR

SEQ ID NO: 110 - protein, 12 aa, synthetic construct
  REGION 1..12: note = source = /note="Description of Artificial Sequence: Synthetic peptide"
EDDIMMAGEFSL

SEQ ID NO: 111 - protein, 12 aa, synthetic construct
  REGION 1..12: note = source = /note="Description of Artificial Sequence: Synthetic peptide"
EDDIMMAGEFGL

SEQ ID NO: 112 - protein, 12 aa, synthetic construct
  REGION 1..12: note = source = /note="Description of Artificial Sequence: Synthetic peptide"
TALVMTDFYFNL

SEQ ID NO: 113 - protein, 11 aa, synthetic construct
  REGION 1..11: note = source = /note="Description of Artificial Sequence: Synthetic peptide"
QASEDIESYLV

SEQ ID NO: 114 - protein, 11 aa, synthetic construct
  REGION 1..11: note = source = /note="Description of Artificial Sequence: Synthetic peptide"
QASQWISNELS

SEQ ID NO: 115 - protein, 7 aa, synthetic construct
  REGION 1..7: note = source = /note="Description of Artificial Sequence: Synthetic peptide"
QASNLAS

SEQ ID NO: 116 - protein, 7 aa, synthetic construct
  REGION 1..7: note = source = /note="Description of Artificial Sequence: Synthetic peptide"
LASTLAS

SEQ ID NO: 117 - protein, 11 aa, synthetic construct
  REGION 1..11: note = source = /note="Description of Artificial Sequence: Synthetic peptide"
QSYVEGGVDVV

SEQ ID NO: 118 - protein, 11 aa, synthetic construct
  REGION 1..11: note = source = /note="Description of Artificial Sequence: Synthetic peptide"
QSYIEGGVDVV

SEQ ID NO: 119 - protein, 12 aa, synthetic construct
  REGION 1..12: note = source = /note="Description of Artificial Sequence: Synthetic peptide"
QQGYNIGHLDNA

SEQ ID NO: 120 - protein, 8 aa, synthetic construct
  REGION 1..8: note = source = /note="Description of Artificial Sequence: Synthetic peptide"
GFSFNLRH

SEQ ID NO: 121 - protein, 8 aa, synthetic construct
  REGION 1..8: note = source = /note="Description of Artificial Sequence: Synthetic peptide"
GFSFSTGY

SEQ ID NO: 122 - protein, 6 aa, synthetic construct
  REGION 1..6: note = source = /note="Description of Artificial Sequence: Synthetic peptide"
HGGSSG

SEQ ID NO: 123 - protein, 6 aa, synthetic construct
  REGION 1..6: note = source = /note="Description of Artificial Sequence: Synthetic peptide"
HGGSSS

SEQ ID NO: 124 - protein, 5 aa, synthetic construct
  REGION 1..5: note = source = /note="Description of Artificial Sequence: Synthetic peptide"
DTGSG

SEQ ID NO: 125 - protein, 12 aa, synthetic construct
  REGION 1..12: note = source = /note="Description of Artificial Sequence: Synthetic peptide"
EDDIMMAGEFSL

SEQ ID NO: 126 - protein, 12 aa, synthetic construct
  REGION 1..12: note = source = /note="Description of Artificial Sequence: Synthetic peptide"
EDDIMMAGEFGL

SEQ ID NO: 127 - protein, 12 aa, synthetic construct
  REGION 1..12: note = source = /note="Description of Artificial Sequence: Synthetic peptide"
TALVMTDFYFNL

SEQ ID NO: 128 - protein, 17 aa, synthetic construct
  REGION 1..17: note = source = /note="Description of Artificial Sequence: Synthetic peptide"
GSTSGSGKPGSGEGSTK

SEQ ID NO: 129 - protein, 6 aa, synthetic construct
  REGION 1..6: note = source = /note="Description of Artificial Sequence: Synthetic peptide"
SGQWMC